European Patent Application EP 4 328 362 A1, published February 28, 2024. Title: Method for Constructing RNA Sequencing Library, Sequencing Method and Kit. Applicant: BGI SHENZHEN. The sequence listing filed with the application follows.

SEQUENCE LISTING (11 sequences)

SEQ ID NO: 1 - DNA, 30 bp, Artificial Sequence
  Synthesized TSO adaptor sequence
  misc_feature (28)..(29): GG is rGrG
  misc_feature (30)..(30): G is modified by LNA
aagcagtggtatcaacgcagagtacatggg

SEQ ID NO: 2 - DNA, 18 bp, Artificial Sequence
  synthesized Tn primer
cgtagccatgtcgttctg

SEQ ID NO: 3 - DNA, 30 bp, Artificial Sequence
  synthesized TSO primer
  misc_feature (1)..(1): 5'Phosphoration
vdcaagcagtggtatcaacgcagagtacat

SEQ ID NO: 4 - DNA, 33 bp, Artificial Sequence
  synthesized TSO-random primer
  misc_feature (1)..(1): 5'phosphoration
  misc_feature (28)..(33): n is a, c, g, or t
aagcagtggtatcaacgcagagtacatnnnnnn

SEQ ID NO: 5 - DNA, 22 bp, Artificial Sequence
  synthesized splint oligo 1
taccactgcttcgtagccatgt

SEQ ID NO: 6 - DNA, 30 bp, Artificial Sequence
  Synthesized poly(A) primer
  misc_feature (1)..(1): 5'phosphoration
aaaaaaaaaaaaaaaaaaaaaaaaaaaaaa

SEQ ID NO: 7 - DNA, 31 bp, Artificial Sequence
  Library adapter
  misc_feature (1)..(1): 5'-Phosphoration
agtcggaggccaagcggtcttaggaagacaa

SEQ ID NO: 8 - DNA, 13 bp, Artificial Sequence
  Library adapter
ttcagcctccggt

SEQ ID NO: 9 - DNA, 30 bp, Artificial Sequence; identical to SEQ ID NO: 6
  Synthesized FP
  misc_feature (1)..(1): 5'-phosphoration

SEQ ID NO: 10 - DNA, 46 bp, Artificial Sequence
  Synthesized RP
  misc_feature (18)..(27): Library index sequence
  misc_feature (18)..(27): Library index sequence, n is a, t, c or g
tgtgagccaaggagttgnnnnnnnnnnttgtcttcctaagaccgct

SEQ ID NO: 11 - DNA, 22 bp, Artificial Sequence
  Synthesized splint oligo 2
ttttttttttttgtgagccaag